European Patent Application EP 4 733 401 A1, published April 29, 2026. Title: 一种利用Cas切口酶制备单链DNA的方法. Applicant: 南京金斯瑞生物科技有限公司. The sequence listing filed with the application follows.

SEQUENCE LISTING (1 sequence)

SEQ ID NO: 1 - DNA, 3553 bp, synthetic construct
  source 1..3553: mol_type = other DNA
taccgttcgtataatgtatgctatacgaacggtactgcagtgtcagccgttaagtgttcctgtgtcactcaaaattgctttgagaggctctaagggcttctcagtgcgttacatccctggcttgttgtccacaaccgttaaaccttaaaagctttaaaagccttatatattcttttttttcttataaaacttaaaaccttagaggctatttaagttgctgatttatattaattttattgttcaaacatgagagcttagtacgtgaaacatgagagcttagtacgttagccatgagagcttagtacgttagccatgagggtttagttcgttaaacatgagagcttagtacgttaaacatgagagcttagtacgtgaaacatgagagcttagtacgtactatcaacaggttgaactgctgatcttcagatcggatccggtttccttgagtggcaggccaggcctggccgtgaacgttcactgaaatcatggcctcttggccaagattgatagcttgtgcctgtccctgagtcccagtccatcacgagcagctggtttctaagatgctatttcccgtataaagcatgagaccgtgacttgccagccccacagagccccgcccttgtccatcactggcatctggactccagcctgggttggggcaaagagggaaatgagatcatgtcctaaccctgatcctcttgtcccacagatatccagaaccctgaccctgccgtggctactaacttcagcctgctgaagcaggctggagacgtggaggagaaccctggacctatggctcttccggtgaccgctcttcttctcccgctggctcttctgctccatgctgcgcgaccggacattcaaatgacccaaactacatcttctttgtctgcttccctgggtgatcgggtgaccatttcatgtagagccagtcaggatataagtaaatacctgaattggtatcaacagaagccagatggaacagtaaagttgctgatttatcacacctcacgattgcactcaggtgttccatccaggttttcaggaagtggctctggaactgactattctttgacaattagtaacttggaacaagaagatattgctacgtatttctgccaacagggtaacactcttccttatacttttggcggcggcactaaattggagattacagggggcggaggctccggtggcggaggatctggcgggggtgggagcgaagttaagttgcaggaaagtgggcctgggttggttgcacccagccaaagcctctcagtaacctgcacggtttccggagtcagtctcccagactacggagtatcatggatccgccagccaccacggaaggggttggagtggctgggagtcatctggggatcagaaacgacgtattacaattccgccctcaaaagccggctgactattataaaagacaacagcaagtcacaagtgttcctgaaaatgaatagtctccagacggatgacacggccatttactattgcgcaaagcactattactacggtgggtcttatgcaatggactactggggtcaagggacctcagtcacagtttccagtactacaactccagcgccgcgacccccgacgccagcaccaacgatagcctctcagccgctttccttgaggccggaggcttgcaggcccgcggccgggggcgcagttcataccagagggcttgattttgcctgtgacatctacatatgggcaccgctcgcaggaacttgtggtgtattgttgctttcactggtgataaccctctattgcaaacgcggacggaagaagctcctctatatttttaagcagccgtttatgcgcccggtacaaacgacgcaggaggaggatggctgttcctgtagatttcctgaagaggaagagggtggatgcgagctcagagtcaaattctcacgctctgcggacgctccagcctacaaacagggtcagaaccagttgtacaacgagcttaatttgggacgccgcgaagagtatgatgtccttgacaaacgcaggggcagggacccggaaatgggcggcaagccacggcgcaagaacccgcaggagggtctgtataacgagcttcagaaggataagatggccgaggcctactcagaaataggaatgaagggagagcggcggagaggcaagggccacgatggtctgtatcaggggctttccacggcaaccaaagacacatatgacgctctccacatgcaggccctccccccgcgggagggcaggggatctctccttacttgtggcgacgtggaggagaaccccggccccagcaagggcgaggagctgttcaccggggtggtgcccatcctggtcgagctggacggcgacgtaaacggccacaagttcagcgtgcgcggcgagggcgagggcgatgccaccaacggcaagctgaccctgaagttcatctgcaccaccggcaagctgcccgtgccctggcccaccctcgtgaccaccctgacctacggcgtgcagtgcttcagccgctaccccgaccacatgaagcgccacgacttcttcaagtccgccatgcccgaaggctacgtccaggagcgcaccatcagcttcaaggacgacggcacctacaagacccgcgccgaggtgaagttcgagggcgacaccctggtgaaccgcatcgagctgaagggcatcgacttcaaggaggacggcaacatcctggggcacaagctggagtacaacttcaacagccacaacgtctatatcaccgccgacaagcagaagaacggcatcaaggccaacttcaagatccgccacaacgtggaggacggcagcgtgcagctcgccgaccactaccagcagaacacccccatcggcgacggccccgtgctgctgcccgacaaccactacctgagcacccagtccgtgctgagcaaagaccccaacgagaagcgcgatcacatggtcctgctggagttcgtgaccgccgccgggatcacttgatgatcataatcaagccatatcacatctgtagaggtttacttgctttaaaaaacctccacacctccccctgaacctgaaacataaaatgaatgcaattgttgttgttaacttgtttattgcagcttataatggttacaaataaagcaatagcatcacaaatttcacaaataaagcatttttttcactgcattctagttgtggtttgtccaaactcatcaatgtatcttatcatgtctggatcaccagctgagagactctaaatccagtgacaagtctgtctgcctattcaccgattttgattctcaaacaaatgtgtcacaaagtaaggattctgatgtgtatatcacagacaaaactgtgctagacatgaggtctatggacttcaagagcaacagtgctgtggcctggagcaacaaatctgactttgcatgtgcaaacgccttcaacaacagcattattccagaagacaccttcttccccagcccaggtaagggcagctttggtgccttcgcaggctgtttccttgcttcaggaatggccatctagagtcgacgcatgc